European Patent Application EP 4 286 410 A1, published December 6, 2023. Title: SINGLE-DOMAIN ANTIBODY AGAINST CD16A AND USE THEREOF. Applicant: Innovent Biologics (Suzhou) Co., Ltd. The sequence listing filed with the application follows.

SEQUENCE LISTING (34 sequences)

SEQ ID NO: 1 - protein, 118 aa, Artificial sequence
  Y88A3 sdAb
EVQLVESGGGLVQPGGSLRLSCAASGYNFTRVYMGWFRQAPGKGREFVAAISWGGGSTHYADSVKGRFTISRDNAKNTLYLQMNSLRAEDTAVYYCALDDYSGVLSPWGQGTLVTVSS

SEQ ID NO: 2 - protein, 120 aa, Artificial sequence
  Y95H1 sdAb
QVQLVESGGGLVQPGGSLRLSCAASGFTFDMYVMTWFRQAPGKGREFVAAIHEDGGKTDYADSVKGRFTISRDNAKNTLYLQMNSLRAEDTAVYYCVAYDYSYSEWYDYWGQGTLVTVSS

SEQ ID NO: 3 - protein, 117 aa, Artificial sequence
  Y99F6 sdAb
QVQLVESGGGLVQPGGSLRLSCAASGFKFNSFVMTWFRQAPGKGREFVAAIHEDGGKTDYADSVKGRFTISRDNAKNTLYLQMNSLRAEDTAVYYCAAVTHSLYDYWGQGTLVTVSS

SEQ ID NO: 4 - protein, 118 aa, Artificial sequence
  Y100D6 sdAb
QVQLVESGGGLVQPGGSLRLSCAASGFTFDWYWMGWFRQAPGKGREFVAAIHDDGTETHYADSVKGRFTISRDNAKNTLYLQMNSLRAEDTAVYYCATVRSDSYYDYWGQGTLVTVSS

SEQ ID NO: 5 - protein, 227 aa, Artificial sequence
  IgG1-Fc-LALA consensus heavy chain sequence
DKTHTCPPCPAPEAAGGPSVFLFPPKPKDTLMISRTPEVTCVVVDVSHEDPEVKFNWYVDGVEVHNAKTKPREEQYNSTYRVVSVLTVLHQDWLNGKEYKCKVSNKALPAPIEKTISKAKGQPREPQVYTLPPSRDELTKNQVSLTCLVKGFYPSDIAVEWESNGQPENNYKTTPPVLDSDGSFFLYSKLTVDKSRWQQGNVFSCSVMHEALHNHYTQKSLSLSPGK

SEQ ID NO: 6 - protein, 120 aa, Artificial sequence
  4LS21 VH
QVQLVQSGAEVKKPGESLKVSCKASGYTFTSYYMHWVRQAPGQGLEWMGAIEPMYGSTSYAQKFQGRVTMTRDTSTSTVYMELSSLRSEDTAVYYCARGSAYYYDFADYWGQGTLVTVSS

SEQ ID NO: 7 - protein, 106 aa, Artificial sequence
  4LS21 VL
SYVLTQPSSVSVAPGQTATISCGGHNIGSKNVHWYQQRPGQSPVLVIYQDNKRPSGIPERFSGSNSGNTATLTISGTQAMDEADYYCQVWDNYSVLFGGGTKLTVL

SEQ ID NO: 8 - protein, 237 aa, Artificial sequence
  CD16A-158V-G129D
MPLLLLLPLLWAGALAMRTEDLPKAVVFLEPQWYRVLEKDSVTLKCQGAYSPEDNSTQWFHNESLISSQASSYFIDAATVDDSGEYRCQTNLSTLSDPVQLEVHIGWLLLQAPRWVFKEEDPIHLRCHSWKNTALHKVTYLQNGKDRKYFHHNSDFYIPKATLKDSGSYFCRGLVGSKNVSSETVNITITQGLAVSTISSFFPPGYQGGGGSGLNDIFEAQKIEWHEGSGSHHHHHH

SEQ ID NO: 9 - protein, 237 aa, Artificial sequence
  CD16A-158V-Y140A
MPLLLLLPLLWAGALAMRTEDLPKAVVFLEPQWYRVLEKDSVTLKCQGAYSPEDNSTQWFHNESLISSQASSYFIDAATVDDSGEYRCQTNLSTLSDPVQLEVHIGWLLLQAPRWVFKEEDPIHLRCHSWKNTALHKVTYLQNGKGRKYFHHNSDFAIPKATLKDSGSYFCRGLVGSKNVSSETVNITITQGLAVSTISSFFPPGYQGGGGSGLNDIFEAQKIEWHEGSGSHHHHHH

SEQ ID NO: 10 - DNA, 6173 bp, Artificial sequence
  Nucleotide sequence of pcDNA3.1 vector
gacggatcgggagatctcccgatcccctatggtgcactctcagtacaatctgctctgatgccgcatagttaagccagtatctgctccctgcttgtgtgttggaggtcgctgagtagtgcgcgagcaaaatttaagctacaacaaggcaaggcttgaccgacaattgcatgaagaatctgcttagggttaggcgttttgcgctgcttcgcgatgtacgggccagatatacgcgttgacattgattattgactagttattaatagtaatcaattacggggtcattagttcatagcccatatatggagttccgcgttacataacttacggtaaatggcccgcctggctgaccgcccaacgacccccgcccattgacgtcaataatgacgtatgttcccatagtaacgccaatagggactttccattgacgtcaatgggtggagtatttacggtaaactgcccacttggcagtacatcaagtgtatcatatgccaagtacgccccctattgacgtcaatgacggtaaatggcccgcctggcattatgcccagtacatgaccttatgggactttcctacttggcagtacatctacgtattagtcatcgctattaccatggtgatgcggttttggcagtacatcaatgggcgtggatagcggtttgactcacggggatttccaagtctccaccccattgacgtcaatgggagtttgttttggcaccaaaatcaacgggactttccaaaatgtcgtaacaactccgccccattgacgcaaatgggcggtaggcgtgtacggtgggaggtctatataagcagagctctctggctaactagagaacccactgcttactggcttatcgaaattaatacgactcactatagggagacccaagctggctagcgtttaaacttaagcttggtaccgagctcggatccactagtccagtgtggtggaattctgcagtcgacggtaccgcgggcccgggatccaccggtcgccaccatggtgagcaagggcgaggagctgttcaccggggtggtgcccatcctggtcgagctggacggcgacgtaaacggccacaagttcagcgtgtccggcgagggcgagggcgatgccacctacggcaagctgaccctgaagttcatctgcaccaccggcaagctgcccgtgccctggcccaccctcgtgaccaccctgacctacggcgtgcagtgcttcagccgctaccccgaccacatgaagcagcacgacttcttcaagtccgccatgcccgaaggctacgtccaggagcgcaccatcttcttcaaggacgacggcaactacaagacccgcgccgaggtgaagttcgagggcgacaccctggtgaaccgcatcgagctgaagggcatcgacttcaaggaggacggcaacatcctggggcacaagctggagtacaactacaacagccacaacgtctatatcatggccgacaagcagaagaacggcatcaaggtgaacttcaagatccgccacaacatcgaggacggcagcgtgcagctcgccgaccactaccagcagaacacccccatcggcgacggccccgtgctgctgcccgacaaccactacctgagcacccagtccgccctgagcaaagaccccaacgagaagcgcgatcacatggtcctgctggagttcgtgaccgccgccgggatcactctcggcatggacgagctgtacaagtaaagcggccgctcgagtctagagggcccgtttaaacccgctgatcagcctcgactgtgccttctagttgccagccatctgttgtttgcccctcccccgtgccttccttgaccctggaaggtgccactcccactgtcctttcctaataaaatgaggaaattgcatcgcattgtctgagtaggtgtcattctattctggggggtggggtggggcaggacagcaagggggaggattgggaagacaatagcaggcatgctggggatgcggtgggctctatggcttctgaggcggaaagaaccagctggggctctagggggtatccccacgcgccctgtagcggcgcattaagcgcggcgggtgtggtggttacgcgcagcgtgaccgctacacttgccagcgccctagcgcccgctcctttcgctttcttcccttcctttctcgccacgttcgccggctttccccgtcaagctctaaatcgggggctccctttagggttccgatttagtgctttacggcacctcgaccccaaaaaacttgattagggtgatggttcacgtagtgggccatcgccctgatagacggtttttcgccctttgacgttggagtccacgttctttaatagtggactcttgttccaaactggaacaacactcaaccctatctcggtctattcttttgatttataagggattttgccgatttcggcctattggttaaaaaatgagctgatttaacaaaaatttaacgcgaattaattctgtggaatgtgtgtcagttagggtgtggaaagtccccaggctccccagcaggcagaagtatgcaaagcatgcatctcaattagtcagcaaccaggtgtggaaagtccccaggctccccagcaggcagaagtatgcaaagcatgcatctcaattagtcagcaaccatagtcccgcccctaactccgcccatcccgcccctaactccgcccagttccgcccattctccgccccatggctgactaattttttttatttatgcagaggccgaggccgcctctgcctctgagctattccagaagtagtgaggaggcttttttggaggcctaggcttttgcaaaaagctcccgggagcttgtatatccattttcggatctgatcaagagacaggatgaggatcgtttcgcatgattgaacaagatggattgcacgcaggttctccggccgcttgggtggagaggctattcggctatgactgggcacaacagacaatcggctgctctgatgccgccgtgttccggctgtcagcgcaggggcgcccggttctttttgtcaagaccgacctgtccggtgccctgaatgaactgcaggacgaggcagcgcggctatcgtggctggccacgacgggcgttccttgcgcagctgtgctcgacgttgtcactgaagcgggaagggactggctgctattgggcgaagtgccggggcaggatctcctgtcatctcaccttgctcctgccgagaaagtatccatcatggctgatgcaatgcggcggctgcatacgcttgatccggctacctgcccattcgaccaccaagcgaaacatcgcatcgagcgagcacgtactcggatggaagccggtcttgtcgatcaggatgatctggacgaagagcatcaggggctcgcgccagccgaactgttcgccaggctcaaggcgcgcatgcccgacggcgaggatctcgtcgtgacccatggcgatgcctgcttgccgaatatcatggtggaaaatggccgcttttctggattcatcgactgtggccggctgggtgtggcggaccgctatcaggacatagcgttggctacccgtgatattgctgaagagcttggcggcgaatgggctgaccgcttcctcgtgctttacggtatcgccgctcccgattcgcagcgcatcgccttctatcgccttcttgacgagttcttctgagcgggactctggggttcgaaatgaccgaccaagcgacgcccaacctgccatcacgagatttcgattccaccgccgccttctatgaaaggttgggcttcggaatcgttttccgggacgccggctggatgatcctccagcgcggggatctcatgctggagttcttcgcccaccccaacttgtttattgcagcttataatggttacaaataaagcaatagcatcacaaatttcacaaataaagcatttttttcactgcattctagttgtggtttgtccaaactcatcaatgtatcttatcatgtctgtataccgtcgacctctagctagagcttggcgtaatcatggtcatagctgtttcctgtgtgaaattgttatccgctcacaattccacacaacatacgagccggaagcataaagtgtaaagcctggggtgcctaatgagtgagctaactcacattaattgcgttgcgctcactgcccgctttccagtcgggaaacctgtcgtgccagctgcattaatgaatcggccaacgcgcggggagaggcggtttgcgtattgggcgctcttccgcttcctcgctcactgactcgctgcgctcggtcgttcggctgcggcgagcggtatcagctcactcaaaggcggtaatacggttatccacagaatcaggggataacgcaggaaagaacatgtgagcaaaaggccagcaaaaggccaggaaccgtaaaaaggccgcgttgctggcgtttttccataggctccgcccccctgacgagcatcacaaaaatcgacgctcaagtcagaggtggcgaaacccgacaggactataaagataccaggcgtttccccctggaagctccctcgtgcgctctcctgttccgaccctgccgcttaccggatacctgtccgcctttctcccttcgggaagcgtggcgctttctcatagctcacgctgtaggtatctcagttcggtgtaggtcgttcgctccaagctgggctgtgtgcacgaaccccccgttcagcccgaccgctgcgccttatccggtaactatcgtcttgagtccaacccggtaagacacgacttatcgccactggcagcagccactggtaacaggattagcagagcgaggtatgtaggcggtgctacagagttcttgaagtggtggcctaactacggctacactagaagaacagtatttggtatctgcgctctgctgaagccagttaccttcggaaaaagagttggtagctcttgatccggcaaacaaaccaccgctggtagcggtttttttgtttgcaagcagcagattacgcgcagaaaaaaaggatctcaagaagatcctttgatcttttctacggggtctgacgctcagtggaacgaaaactcacgttaagggattttggtcatgagattatcaaaaaggatcttcacctagatccttttaaattaaaaatgaagttttaaatcaatctaaagtatatatgagtaaacttggtctgacagttaccaatgcttaatcagtgaggcacctatctcagcgatctgtctatttcgttcatccatagttgcctgactccccgtcgtgtagataactacgatacgggagggcttaccatctggccccagtgctgcaatgataccgcgagacccacgctcaccggctccagatttatcagcaataaaccagccagccggaagggccgagcgcagaagtggtcctgcaactttatccgcctccatccagtctattaattgttgccgggaagctagagtaagtagttcgccagttaatagtttgcgcaacgttgttgccattgctacaggcatcgtggtgtcacgctcgtcgtttggtatggcttcattcagctccggttcccaacgatcaaggcgagttacatgatcccccatgttgtgcaaaaaagcggttagctccttcggtcctccgatcgttgtcagaagtaagttggccgcagtgttatcactcatggttatggcagcactgcataattctcttactgtcatgccatccgtaagatgcttttctgtgactggtgagtactcaaccaagtcattctgagaatagtgtatgcggcgaccgagttgctcttgcccggcgtcaatacgggataataccgcgccacatagcagaactttaaaagtgctcatcattggaaaacgttcttcggggcgaaaactctcaaggatcttaccgctgttgagatccagttcgatgtaacccactcgtgcacccaactgatcttcagcatcttttactttcaccagcgtttctgggtgagcaaaaacaggaaggcaaaatgccgcaaaaaagggaataagggcgacacggaaatgttgaatactcatactcttcctttttcaatattattgaagcatttatcagggttattgtctcatgagcggatacatatttgaatgtatttagaaaaataaacaaataggggttccgcgcacatttccccgaaaagtgccacctgacgtc

SEQ ID NO: 11 - DNA, 6934 bp, Artificial sequence
  Nucleotide sequence of pXC17.4 vector
gaattcattgatcataatcagccataccacatttgtagaggttttacttgctttaaaaaacctcccacacctccccctgaacctgaaacataaaatgaatgcaattgttgttgttaacttgtttattgcagcttataatggttacaaataaagcaatagcatcacaaatttcacaaataaagcatttttttcactgcattctagttgtggtttgtccaaactcatcaatgtatcttatcatgtctggcggccgcgacctgcaggcgcagaactggtaggtatggaagatccctcgagatccattgtgctggcggtaggcgagcagcgcctgcctgaagctgcgggcattcccgatcagaaatgagcgccagtcgtcgtcggctctcggcaccgaatgcgtatgattctccgccagcatggcttcggccagtgcgtcgagcagcgcccgcttgttcctgaagtgccagtaaagcgccggctgctgaacccccaaccgttccgccagtttgcgtgtcgtcagaccgtctacgccgacctcgttcaacaggtccagggcggcacggatcactgtattcggctgcaactttgtcatgcttgacactttatcactgataaacataatatgtccaccaacttatcagtgataaagaatccgcgccagcacaatggatctcgaggtcgagggatctctagaggatcctctacgccggacgcatcgtggccggcatcaccggcgccacaggtgcggttgctggcgcctatatcgccgacatcaccgatggggaagatcgggctcgccacttcgggctcatgagcgcttgtttcggcgtgggtatggtggcaggccccgtggccgggggactgttgggcgccatctccttgcatgcaccattccttgcggcggcggtgctcaacggcctcaacctactactgggctgcttcctaatgcaggagtcgcataagggagagcgtcgacctcgggccgcgttgctggcgtttttccataggctccgcccccctgacgagcatcacaaaaatcgacgctcaagtcagaggtggcgaaacccgacaggactataaagataccaggcgtttccccctggaagctccctcgtgcgctctcctgttccgaccctgccgcttaccggatacctgtccgcctttctcccttcgggaagcgtggcgctttctcatagctcacgctgtaggtatctcagttcggtgtaggtcgttcgctccaagctgggctgtgtgcacgaaccccccgttcagcccgaccgctgcgccttatccggtaactatcgtcttgagtccaacccggtaagacacgacttatcgccactggcagcagccactggtaacaggattagcagagcgaggtatgtaggcggtgctacagagttcttgaagtggtggcctaactacggctacactagaagaacagtatttggtatctgcgctctgctgaagccagttaccttcggaaaaagagttggtagctcttgatccggcaaacaaaccaccgctggtagcggtggtttttttgtttgcaagcagcagattacgcgcagaaaaaaaggatctcaagaagatcctttgatcttttctacggggtctgacgctcagtggaacgaaaactcacgttaagggattttggtcatgagattatcaaaaaggatcttcacctagatccttttaaattaaaaatgaagttttaaatcaatctaaagtatatatgagtaaacttggtctgacagttaccaatgcttaatcagtgaggcacctatctcagcgatctgtctatttcgttcatccatagttgcctgactccccgtcgtgtagataactacgatacgggagggcttaccatctggccccagtgctgcaatgataccgcgagacccacgctcaccggctccagatttatcagcaataaaccagccagccggaagggccgagcgcagaagtggtcctgcaactttatccgcctccatccagtctattaattgttgccgggaagctagagtaagtagttcgccagttaatagtttgcgcaacgttgttgccattgctacaggcatcgtggtgtcacgctcgtcgtttggtatggcttcattcagctccggttcccaacgatcaaggcgagttacatgatcccccatgttgtgcaaaaaagcggttagctccttcggtcctccgatcgttgtcagaagtaagttggccgcagtgttatcactcatggttatggcagcactgcataattctcttactgtcatgccatccgtaagatgcttttctgtgactggtgagtactcaaccaagtcattctgagaatagtgtatgcggcgaccgagttgctcttgcccggcgtcaatacgggataataccgcgccacatagcagaactttaaaagtgctcatcattggaaaacgttcttcggggcgaaaactctcaaggatcttaccgctgttgagatccagttcgatgtaacccactcgtgcacccaactgatcttcagcatcttttactttcaccagcgtttctgggtgagcaaaaacaggaaggcaaaatgccgcaaaaaagggaataagggcgacacggaaatgttgaatactcatactcttcctttttcaatattattgaagcatttatcagggttattgtctcatgagcggatacatatttgaatgtatttagaaaaataaacaaataggggttccgcgcacatttccccgaaaagtgccacctgacgtctaagaaaccattattatcatgacattaacctataaaaataggcgtatcacgaggccctgatggctctttgcggcacccatcgttcgtaatgttccgtggcaccgaggacaaccctcaagagaaaatgtaatcacactggctcaccttcgggtgggcctttctgcgtttataaggagacactttatgtttaagaaggttggtaaattccttgcggctttggcagccaagctagatccggctgtggaatgtgtgtcagttagggtgtggaaagtccccaggctccccagcaggcagaagtatgcaaagcatgcatctcaattagtcagcaaccaggtgtggaaagtccccaggctccccagcaggcagaagtatgcaaagcatgcatctcaattagtcagcaaccatagtcccgcccctaactccgcccatcccgcccctaactccgcccagttccgcccattctccgccccatggctgactaattttttttatttatgcagaggccgaggccgcctcggcctctgagctattccagaagtagtgaggaggcttttttggaggcctaggcttttgcaaaaagctagcttggggccaccgctcagagcaccttccaccatggccacctcagcaagttcccacttgaacaaaaacatcaagcaaatgtacttgtgcctgccccagggtgagaaagtccaagccatgtatatctgggttgatggtactggagaaggactgcgctgcaaaacccgcaccctggactgtgagcccaagtgtgtagaagagttacctgagtggaattttgatggctctagtacctttcagtctgagggctccaacagtgacatgtatctcagccctgttgccatgtttcgggaccccttccgcagagatcccaacaagctggtgttctgtgaagttttcaagtacaaccggaagcctgcagagaccaatttaaggcactcgtgtaaacggataatggacatggtgagcaaccagcacccctggtttggaatggaacaggagtatactctgatgggaacagatgggcacccttttggttggccttccaatggctttcctgggccccaaggtccgtattactgtggtgtgggcgcagacaaagcctatggcagggatatcgtggaggctcactaccgcgcctgcttgtatgctggggtcaagattacaggaacaaatgctgaggtcatgcctgcccagtgggagttccaaataggaccctgtgaaggaatccgcatgggagatcatctctgggtggcccgtttcatcttgcatcgagtatgtgaagactttggggtaatagcaacctttgaccccaagcccattcctgggaactggaatggtgcaggctgccataccaactttagcaccaaggccatgcgggaggagaatggtctgaagcacatcgaggaggccatcgagaaactaagcaagcggcaccggtaccacattcgagcctacgatcccaaggggggcctggacaatgcccgtcgtctgactgggttccacgaaacgtccaacatcaacgacttttctgctggtgtcgccaatcgcagtgccagcatccgcattccccggactgtcggccaggagaagaaaggttactttgaagaccgccgcccctctgccaattgtgacccctttgcagtgacagaagccatcgtccgcacatgccttctcaatgagactggcgacgagcccttccaatacaaaaactaattagactttgagtgatcttgagcctttcctagttcatcccaccccgccccagagagatctttgtgaaggaaccttacttctgtggtgtgacataattggacaaactacctacagagatttaaagctctaaggtaaatataaaatttttaagtgtataatgtgttaaactactgattctaattgtttgtgtattttagattccaacctatggaactgatgaatgggagcagtggtggaatgcctttaatgaggaaaacctgttttgctcagaagaaatgccatctagtgatgatgaggctactgctgactctcaacattctactcctccaaaaaagaagagaaaggtagaagaccccaaggactttccttcagaattgctaagttttttgagtcatgctgtgtttagtaatagaactcttgcttgctttgctatttacaccacaaaggaaaaagctgcactgctatacaagaaaattatggaaaaatattctgtaacctttataagtaggcataacagttataatcataacatactgttttttcttactccacacaggcatagagtgtctgctattaataactatgctcaaaaattgtgtacctttagctttttaatttgtaaaggggttaataaggaatatttgatgtatagtgccttgactagagatcataatcagccataccacatttgtagaggttttacttgctttaaaaaacctcccacacctccccctgaacctgaaacataaaatgaatgcaattgttgttgttaacttgtttattgcagcttataatggttacaaataaagcaatagcatcacaaatttcacaaataaagcatttttttcactgcattctagttgtggtttgtccaaactcatcaatgtatcttatcatgtctggatctctagcttcgtgtcaaggacggtgaggcgcgcctactgagtcattagggactttccaatgggttttgcccagtacataaggtcaataggggtgaatcaacaggaaagtcccattggagccaagtacactgagtcaatagggactttccattgggttttgcccagtacaaaaggtcaatagggggtgagtcaatgggtttttcccattattggcacgtacataaggtcaataggggtgagtcattgggtttttccagccaatttaattaaaacgccatgtactttcccaccattgacgtcaatgggctattgaaactaatgcaacgtgacctttaaacggtactttcccatagctgattaatgggaaagtaccgttctcgagccaatacacgtcaatgggaagtgaaagggcagccaaaacgtaacaccgccccggttttcccctggaaattccatattggcacgcattctattggctgagctgcgttctacgtgggtataagaggcgcgaccagcgtcggtaccgtcgcagtcttcggtctgaccaccgtagaacgcagcctcaggacctccatagaagacaccgggaccgatccagcctccgcggccgggaacggtgcattggaacgcggattccccgtgccaagagtgacgtaagtaccgcctatagagtctataggcccacccccttggcttcttatgcatgctatactgtttttggcttggggtctatacacccccgcttcctcatgttataggtgatggtatagcttagcctataggtgtgggttattgaccattattgaccactcccctattggtgacgatactttccattactaatccataacatggctctttgccacaactctctttattggctatatgccaatacactgtccttcagagactgacacggactctgtatttttacaggatggggtctcatttattatttacaaattcacatatacaacaccaccgtccccagtgcccgcagtttttattaaacataacgtgggatctccacgcgaatctcgggtacgtgttccggacatgggctcttctccggtagcggcggagcttctacatccgagccctgctcccatgcctccagcgactcatggtcgctcggcagctccttgctcctaacagtggaggccagacttaggcacagcacgatgcccaccaccaccagtgtgccgcacaaggccgtggcggtagggtatgtgtctgaaaatgagctcggggagcgggcttgcaccgctgacgcatttggaagacttaaggcagcggcagaagaagatgcaggcagctgagttgttgtgttctgataagagtcagaggtaactcccgttgcggtgctgttaacggtggagggcagtgtagtctgagcagtactcgttgctgccgcgcgcgccaccagacataatagctgacagactaacagactgttcctttccatgggtcttttctgcagtcaccgtccttgacacgaagcttcgcgacgtacgttcgaacccgggcacgtgcggacc

SEQ ID NO: 12 - protein, 119 aa, Artificial sequence
  Anti-HEL antibody VH
EVRLLESGGGLVQPGGSLRLSCAASGFTFSNYAMGWVRQAPGKCLEWVSAISGSGGSTYYADSVKGRFTTSRDDSKNALYLQMNSLRAEDTAVYYCARGGPGWYAADVWGQGTTVTVSS

SEQ ID NO: 13 - protein, 107 aa, Artificial sequence
  Anti-HEL antibody VL
DIQMTQSPSSLSASVGDRVTITCRASQSISSYLNWYQQKPGKAPKLLIYAASSLQSGVPSRFSGSGSGTDFTLTISSLQPEDFATYYCQQADLPAFAFGCGTKVEIK

SEQ ID NO: 14 - protein, 227 aa, Artificial sequence
  IgG1-LALA-Fc-Knob
DKTHTCPPCPAPEAAGGPSVFLFPPKPKDTLMISRTPEVTCVVVDVSHEDPEVKFNWYVDGVEVHNAKTKPREEQYNSTYRVVSVLTVLHQDWLNGKEYKCKVSNKALPAPIEKTISKAKGQPREPQVYTLPPCRDELTKNQVSLWCLVKGFYPSDIAVEWESNGQPENNYKTTPPVLDSDGSFFLYSKLTVDKSRWQQGNVFSCSVMHEALHNHYTQKSLSLSPGK

SEQ ID NO: 15 - protein, 120 aa, Artificial sequence [sequence omitted]

SEQ ID NO: 16 - protein, 107 aa, Artificial sequence [sequence omitted]

SEQ ID NO: 17 - protein, 124 aa, Artificial sequence
  Anti-BCMA antibody clone ADI384-56 VH
EVQLVESGGGLVQPGRSLRLSCAASGFTFGDYAIHWVRQAPGKGLEWVSGISWDSSSIAYADSVKGRFTISRDNAKNSLYLQMNSLRAEDTAVYYCAKDSPVRDSFGSIAFDIWGQGTMVTVSS

SEQ ID NO: 18 - protein, 107 aa, Artificial sequence
  Anti-BCMA antibody clone ADI384-56 VL
EIVLTQSPATLSLSPGERATLSCRASQSVSSYLAWYQQKPGQAPRLLIYDASKRATGIPARFSGSGSGTDFTLTISSLEPEDFAVYYCQQASALPLTFGGGTKVEIK

SEQ ID NO: 19 - protein, 330 aa, Artificial sequence
  IgG1-LALA-CH-Hole
ASTKGPSVFPLAPSSKSTSGGTAALGCLVKDYFPEPVTVSWNSGALTSGVHTFPAVLQSSGLYSLSSVVTVPSSSLGTQTYICNVNHKPSNTKVDKKVEPKSCDKTHTCPPCPAPEAAGGPSVFLFPPKPKDTLMISRTPEVTCVVVDVSHEDPEVKFNWYVDGVEVHNAKTKPREEQYNSTYRVVSVLTVLHQDWLNGKEYKCKVSNKALPAPIEKTISKAKGQPREPQVCTLPPSRDELTKNQVSLSCAVKGFYPSDIAVEWESNGQPENNYKTTPPVLDSDGSFFLVSKLTVDKSRWQQGNVFSCSVMHEALHNHYTQKSLSLSPGK

SEQ ID NO: 20 - protein, 107 aa, Artificial sequence [sequence omitted]

SEQ ID NO: 21 - protein, 450 aa, Artificial sequence
  Margetuximab or MGAH22, HC
QVQLQQSGPELVKPGASLKLSCTASGFNIKDTYIHWVKQRPEQGLEWIGRIYPTNGYTRYDPKFQDKATITADTSSNTAYLQVSRLTSEDTAVYYCSRWGGDGFYAMDYWGQGASVTVSSASTKGPSVFPLAPSSKSTSGGTAALGCLVKDYFPEPVTVSWNSGALTSGVHTFPAVLQSSGLYSLSSVVTVPSSSLGTQTYICNVNHKPSNTKVDKRVEPKSCDKTHTCPPCPAPELVGGPSVFLLPPKPKDTLMISRTPEVTCVVVDVSHEDPEVKFNWYVDGVEVHNAKTKPPEEQYNSTLRVVSVLTVLHQDWLNGKEYKCKVSNKALPAPIEKTISKAKGQPREPQVYTLPPSRDELTKNQVSLTCLVKGFYPSDIAVEWESNGQPENNYKTTPLVLDSDGSFFLYSKLTVDKSRWQQGNVFSCSVMHEALHNHYTQKSLSLSPGK

SEQ ID NO: 22 - protein, 107 aa, Artificial sequence
  Margetuximab or MGAH22 VL
DIVMTQSHKFMSTSVGDRVSITCKASQDVNTAVAWYQQKPGHSPKLLIYSASFRYTGVPDRFTGSRSGTDFTFTISSVQAEDLAVYYCQQHYTTPPTFGGGTKVEIK

SEQ ID NO: 23 - protein, 9 aa, Artificial sequence
  Y88A3 CDR1 (Kabat numbering)
YNFTRVYMG

SEQ ID NO: 24 - protein, 10 aa, Artificial sequence
  Y88A3 CDR2 (Kabat numbering)
AISWGGGSTH

SEQ ID NO: 25 - protein, 11 aa, Artificial sequence
  Y88A3 CDR3 (Kabat numbering)
ALDDYSGVLSP

SEQ ID NO: 26 - protein, 9 aa, Artificial sequence
  Y95H1 CDR1 (Kabat numbering)
FTFDMYVMT

SEQ ID NO: 27 - protein, 10 aa, Artificial sequence
  Y95H1 CDR2 (Kabat numbering)
AIHEDGGKTD

SEQ ID NO: 28 - protein, 13 aa, Artificial sequence
  Y95H1 CDR3 (Kabat numbering)
VAYDYSYSEWYDY

SEQ ID NO: 29 - protein, 9 aa, Artificial sequence
  Y99F6 CDR1 (Kabat numbering)
FKFNSFVMT

SEQ ID NO: 30 - protein, 10 aa, Artificial sequence
  Y99F6 CDR2 (Kabat numbering)
AIHEDGGKTD

SEQ ID NO: 31 - protein, 10 aa, Artificial sequence
  Y99F6 CDR3 (Kabat numbering)
AAVTHSLYDY

SEQ ID NO: 32 - protein, 9 aa, Artificial sequence
  Y100D6 CDR1 (Kabat numbering)
FTFDWYWMG

SEQ ID NO: 33 - protein, 10 aa, Artificial sequence
  Y100D6 CDR2 (Kabat numbering)
AIHDDGTETH

SEQ ID NO: 34 - protein, 11 aa, Artificial sequence
  Y100D6 CDR3 (Kabat numbering)
ATVRSDSYYDY